European Patent Application EP 4 512 895 A1, published February 26, 2025. Title: Fructanase variants. Applicant: AB Enzymes Oy. The sequence listing filed with the application follows.

SEQUENCE LISTING (7 sequences)

SEQ ID NO: 1 - protein, 1279 aa, Lactobacillus crispatus
DTQSPVNIEQKNKSAELIKQNSDISTSAQQHNKNANGKTEDTSTQSTSTDLQNTNGKTEDTSTQSTSTDLQNTNTQKSFKNQSQEPESSTKAGEVKTLKDFTFSQNGKWSEQKDGIHSDARGQGDSFAYTKVKGDNFMYSADVVFQTNQGAAAITFRDNNDPDNKDGYAVNVDASSHKAKFWRWHDNKDYQLIDERDVKQTADNTYNLKVVANGHWLEYFVNDVLVASNGDYTLQKGDKGQPSVTNNGYFGLLNWNSNVIFKNVKYTKLDQSFTPLVSDITVTSDKGKVEEKGQFSPEQPIYIQYVDNDASTVNLKVKTDSPKAKVVAYDLNNNAYTDLKNIPVQVGANYLTVVSEVTASDGTKVESVYRINVHRLHPNENYYNELYRDQYHFSVKEGWSNDPNGLVYFNGKYHMFYQFYDDTIWGPMHWAHATSKDLIHWKNEPIALYPDANGAMFSGSIVVDKGNTSGLFDNDKGGLVALVTTDGNGQRIELAYSRDEGKTWDKLPNLVADWQKDPLQVQDFRDPKVFRWNDKWFMVLAGGPLRIYSSTNLQNWQVESEYSNINTECPDLYPIRANDGQLKWVLSRGGRFYKIGDFKEVNGKWSFIPDEAYKDQDGIMNFGKDSYAAMTYYQHSFGTEKDPTLPDIIEENWMNNWDYCNLVGNTVGQSFNGTYNLNLKVGLVKDGDKYLLTQTPIKAYEALRDNAHKVEYKDVTVTPNNDLFKNFKGDSYEIVSTFRPSKSTTKVGFNVRVGKGQATKVIYDLTTNKIYIDRSKSGVQINNKFSELNEQPVTRNADGSISLHLYVDRASVEAFTKGDTVLGANQIFPAPQSLGLQVVSEGGDSKADITLYPIKSVWTDKQKVNKPLEIVQVSPKEVRLNVGDSTTLTAYVMPGNVSQALDWSINDESLASITKDPESNSLKIVAKKAGTLTVTVKSHEDPSLSKTYKITILKNNFKTNIKDLKPLSGNWYVDDQDLHDENVSSNDYIMSPTKVSSSEYDMNLDVKYQKGLVNIFFASANEDPNGAYSLQLGGDKTLRLFRFYGDTITTTDLPAALNDGKLHHVAIHKTQNAVKVTIDGKEAMDYTFDKVDPGFNSAYVGLGLWDGAADFQNLYVKAATENDDNSSSSIDFNDQEIPNVSTDDNNSIIEKPSETVKTVVFTAKSLMHNAFVYDNQGKRIEKIVLKAGSVLKVGHIKLINHKRYYQLDNGKYIKAGNIDAYVRKLRRNAFVYNRAGKHIKKSLIRKGKKVKTYGSPVVIKGIKYYIVGNNRYIKAVNFM

SEQ ID NO: 2 - protein, 1165 aa, synthetic construct
DTQSPVNIEQKNKSAELIKQNSDISTSAQQHNKNANGKTEDTSTQSTSTDLQNTNGKTEDTSTQSTSTDLQNTNTQKSFKNQSQEPESSTKAGEVKTLKDFTFSQNGKWSEQKDGIHSDARGQGDSFAYTKVKGDNFMYSADVVFQTNQGAAAITFRDNNDPDNKDGYAVNVDASSHKAKFWRWHDNKDYQLIDERDVKQTADNTYNLKVVANGHWLEYFVNDVLVASNGDYTLQKGDKGQPSVTNNGYFGLLNWNSNVIFKNVKYTKLDQSFTPLVSDITVTSDKGKVEEKGQFSPEQPIYIQYVDNDASTVNLKVKTDSPKAKVVAYDLNNNAYTDLKNIPVQVGANYLTVVSEVTASDGTKVESVYRINVHRLHPNENYYNELYRDQYHFSVKEGWSNDPNGLVYFNGKYHMFYQFYDDTIWGPMHWAHATSKDLIHWKNEPIALYPDANGAMFSGSIVVDKGNTSGLFDNDKGGLVALVTTDGNGQRIELAYSRDEGKTWDKLPNLVADWQKDPLQVQDFRDPKVFRWNDKWFMVLAGGPLRIYSSTNLQNWQVESEYSNINTECPDLYPIRANDGQLKWVLSRGGRFYKIGDFKEVNGKWSFIPDEAYKDQDGIMNFGKDSYAAMTYYQHSFGTEKDPTLPDIIEENWMNNWDYCNLVGNTVGQSFNGTYNLNLKVGLVKDGDKYLLTQTPIKAYEALRDNAHKVEYKDVTVTPNNDLFKNFKGDSYEIVSTFRPSKSTTKVGFNVRVGKGQATKVIYDLTTNKIYIDRSKSGVQINNKFSELNEQPVTRNADGSISLHLYVDRASVEAFTKGDTVLGANQIFPAPQSLGLQVVSEGGDSKADITLYPIKSVWTDKQKVNKPLEIVQVSPKEVRLNVGDSTTLTAYVMPGNVSQALDWSINDESLASITKDPESNSLKIVAKKAGTLTVTVKSHEDPSLSKTYKITILKNNFKTNIKDLKPLSGNWYVDDQDLHDENVSSNDYIMSPTKVSSSEYDMNLDVKYQKGLVNIFFASANEDPNGAYSLQLGGDKTLRLFRFYGDTITTTDLPAALNDGKLHHVAIHKTQNAVKVTIDGKEAMDYTFDKVDPGFNSAYVGLGLWDGAADFQNLYVKAATENDDNSSSSIDFNDQEIPNVSTDDNNSIIEKPSETVKTVVFTAKS

SEQ ID NO: 3 - DNA, 22 bp, synthetic construct
  source 1..22: mol_type = other DNA
gtttcctctccctctcattttc

SEQ ID NO: 4 - DNA, 21 bp, synthetic construct
  source 1..21: mol_type = other DNA
taaagagatataccgacagtg

SEQ ID NO: 5 - DNA, 44 bp, synthetic construct
  source 1..44: mol_type = other DNA
atgagagggagaggaaacatgagtcataaatttaataattacgg

SEQ ID NO: 6 - DNA, 35 bp, synthetic construct
  source 1..35: mol_type = other DNA
ggtatatctctttaagactttgccgtaaagacaac

SEQ ID NO: 7 - DNA, 40 bp, synthetic construct
  source 1..40: mol_type = other DNA
ggtatatctctttacataaagttaaccgctttaatatatc